European Patent Specification EP 3 651 785 B1, published November 12, 2025. Title: COMPOSITIONS AND METHODS FOR TREATING MYELIN DISORDERS. Applicant: CASE WESTERN RESERVE UNIVERSITY SILVER, Jerry. The sequence listing filed with the application follows.

SEQUENCE LISTING (62 sequences)

SEQ ID NO: 1 - protein, 22 aa, Xenopus borealis
DLAEHTEHLKANDNLKSQEYES

SEQ ID NO: 2 - protein, 22 aa, Anolis carolinensis
DHTEHELKANDNLKLSQEYESI

SEQ ID NO: 3 - protein, 24 aa, Danio rerio
ELAEHTELLKANDNLKLSQEYESI

SEQ ID NO: 4 - protein, 24 aa, Oreochromis aureus
ELAEHTELLKANDNLKLSQEYESI

SEQ ID NO: 5 - protein, 24 aa, Gallus gallus
ELAEHTEHLKANDNLKLSQEYESI

SEQ ID NO: 6 - protein, 24 aa, Fringilla coelebs
ELAEHTEHLKANDNLKLSQEYESI

SEQ ID NO: 7 - protein, 24 aa, Ornithorhynchus anatinus
ELAEHTDHLKANDNLKLSQEYESI

SEQ ID NO: 8 - protein, 24 aa, Sarcophilus harrisii
EMAEHTEHLKANDNLKLSQEYESI

SEQ ID NO: 9 - protein, 24 aa, Mustela putorius
DMAEHTERLKANDSLKLSQEYESI

SEQ ID NO: 10 - protein, 24 aa, Galago alleni
DMAEHTERLKANDSLKLSQEYESI

SEQ ID NO: 11 - protein, 24 aa, Callithrix aurita
DMAEHTERLKANDSLKLSQEYESI

SEQ ID NO: 12 - protein, 24 aa, Rattus rattus
DMAEHMERLKANDSLKLSQEYESI

SEQ ID NO: 13 - protein, 24 aa, Mus musculus
DMAEHMERLKANDSLKLSQEYESI

SEQ ID NO: 14 - protein, 24 aa, Canis familiaris
DMAEHTERLKANDSLKLSQEYESI

SEQ ID NO: 15 - protein, 24 aa, Sus barbatus
DMAEHTERLKANDSLKLSQEYESI

SEQ ID NO: 16 - protein, 24 aa, Bos primigenius
DMAEHTERLKANDSLKLSQEYESI

SEQ ID NO: 17 - protein, 24 aa, Ovis aries
DMAEHTERLKANDSLKLSQEYESI

SEQ ID NO: 18 - protein, 24 aa, Orcinus orca
DMAEHTERLKANDSLKLSQEYESI

SEQ ID NO: 19 - protein, 24 aa, Saimiri sciureus
DMAEHTERLKANDSLKLSQEYESI

SEQ ID NO: 20 - protein, 24 aa, Papio hamadryas
DMAEHTERLKANDSLKLSQEYESI

SEQ ID NO: 21 - protein, 24 aa, Primate calicivirus
DMAEHTERLKANDSLKLSQEYESI

SEQ ID NO: 22 - protein, 24 aa, Primate calicivirus
DMAEHTERLKANDSLKLSQEYESI

SEQ ID NO: 23 - protein, 24 aa, Macaca radiata
DMAEHTERLKANDSLKLSQEYESI

SEQ ID NO: 24 - protein, 24 aa, Pan troglodytes
DMAEHTERLKANDSLKLSQEYESI

SEQ ID NO: 25 - protein, 24 aa, Homo sapiens
DMAEHTERLKANDSLKLSQEYESI

SEQ ID NO: 26 - protein, 24 aa, Rattus rattus
DLADNIERLKANDGLKFSQEYESI

SEQ ID NO: 27 - protein, 24 aa, Rattus rattus
ELADHIERLKANDNLKFSQEYESI

SEQ ID NO: 28 - protein, 24 aa, Rattus rattus
KLEEEINRRMADDNKIFREEFNAL

SEQ ID NO: 29 - protein, 10 aa, Homo sapiens
DMAEHTERLK

SEQ ID NO: 30 - protein, 4 aa, Homo sapiens
ANDS

SEQ ID NO: 31 - protein, 10 aa, Homo sapiens
LKLSQEYESI

SEQ ID NO: 32 - protein, 14 aa, Artificial Sequence
  Synthetic Construct
  MISC_FEATURE (3)..(3): Xaa is Thr or Met
EHXERLKANDSLKL

SEQ ID NO: 33 - protein, 14 aa, Artificial Sequence
  Synthetic Construct
  misc_feature (6)..(6): Xaa can be any naturally occurring amino acid
DMAEHXERLKANDS

SEQ ID NO: 34 - protein, 33 aa, Xenopus borealis
GRKKRRQRRRCDLAEHTEHLKANDNLKSQEYES

SEQ ID NO: 35 - protein, 32 aa, Anolis carolinensis
GRKKRRQRRRCDHTEHLKANDNLKLSQEYESI

SEQ ID NO: 36 - protein, 35 aa, Danio rerio
GRKKRRQRRRCELAEHTELLKANDNLKLSQEYESI

SEQ ID NO: 37 - protein, 35 aa, Tilapia nilotica; identical to SEQ ID NO: 36

SEQ ID NO: 38 - protein, 35 aa, Gallus gallus
GRKKRRQRRRCELAEHTEHLKANDNLKLSQEYESI

SEQ ID NO: 39 - protein, 35 aa, Fringilla coelebs; identical to SEQ ID NO: 38

SEQ ID NO: 40 - protein, 35 aa, Ornithorhynchus anatinus
GRKKRRQRRRCELAEHTDHLKANDNLKLSQEYESI

SEQ ID NO: 41 - protein, 35 aa, Sarcophilus harrisii
GRKKRRQRRRCEMAEHTEHLKANDNLKLSQEYESI

SEQ ID NO: 42 - protein, 35 aa, Mustela putorius
GRKKRRQRRRCDMAEHTERLKANDSLKLSQEYESI

SEQ ID NO: 43 - protein, 35 aa, Galago alleni; identical to SEQ ID NO: 42

SEQ ID NO: 44 - protein, 35 aa, Callithrix argentata; identical to SEQ ID NO: 42

SEQ ID NO: 45 - protein, 35 aa, Rattus rattus
GRKKRRQRRRCDMAEHMERLKANDSLKLSQEYESI

SEQ ID NO: 46 - protein, 35 aa, Mus musculus; identical to SEQ ID NO: 45

SEQ ID NO: 47 - protein, 35 aa, Canis familiaris; identical to SEQ ID NO: 42

SEQ ID NO: 48 - protein, 35 aa, Sus barbatus; identical to SEQ ID NO: 42

SEQ ID NO: 49 - protein, 35 aa, Bos primigenius; identical to SEQ ID NO: 42

SEQ ID NO: 50 - protein, 35 aa, Ovis aries; identical to SEQ ID NO: 42

SEQ ID NO: 51 - protein, 35 aa, Orcinus orca; identical to SEQ ID NO: 42

SEQ ID NO: 52 - protein, 35 aa, Saimiri boliviensis; identical to SEQ ID NO: 42

SEQ ID NO: 53 - protein, 35 aa, Papio hamadryas; identical to SEQ ID NO: 42

SEQ ID NO: 54 - protein, 35 aa, Primate calicivirus; identical to SEQ ID NO: 42

SEQ ID NO: 55 - protein, 35 aa, Primate calicivirus; identical to SEQ ID NO: 42

SEQ ID NO: 56 - protein, 35 aa, Macaca arctoides; identical to SEQ ID NO: 42

SEQ ID NO: 57 - protein, 35 aa, Pan troglodytes; identical to SEQ ID NO: 42

SEQ ID NO: 58 - protein, 35 aa, Homo sapiens; identical to SEQ ID NO: 42

SEQ ID NO: 59 - protein, 25 aa, Artificial Sequence
  Synthetic Construct
  MISC_FEATURE (14)..(14): Xaa is Thr or Met
GRKKRRQRRRCEHXERLKANDSLKL

SEQ ID NO: 60 - protein, 25 aa, Artificial Sequence
  Synthetic Construct
  MISC_FEATURE (17)..(17): X1 is T or M
GRKKRRQRRRCDMAEHXERLKANDS

SEQ ID NO: 61 - protein, 35 aa, Artificial Sequence; identical to SEQ ID NO: 45
  Synthetic Construct
  MISC_FEATURE: X1 is T or M
  MISC_FEATURE (17)..(17): X1 is T or M

SEQ ID NO: 62 - protein, 35 aa, Artificial Sequence
  Synthetic Construct
GRKKRRQRRRCIREDDSLMLYALAQEKKESNMHES